European Patent Application EP 4 488 375 A1, published January 8, 2025. Title: Verfahren zur Herstellung einer wässrigen Lösung enthaltend Allose. Applicant: Annikki GmbH. Application EP. The sequence listing filed with the application follows.

SEQUENCE LISTING (18 sequences)

SEQ ID NO: 1 - protein, 325 aa, Thermochaetoides thermophila
MAPQIPNIKLSSGYDMPQVGFGLWKVDRSICADVVYNAIKIGYRLFDGACDYGNEVEAGQGIARAIKEGIVKREELFIVSKLWNTFHDGDKVEPIVRKQLADWGIDYFDLYLVHFPVALEYVDPSVRYPPGWFYDGEKEIRPSKATIQETWTAMESLVEKGLARSIGVSNFQAQLLYDLLRYAKIRPATLQIEHHPFLVQQELLNLAKAEGIAVTAYSSFGPQSFLEFNMKHAVQLTPLFEDETIKKIAAKYNRPASQVLLRWATQRGLAIIPKSTRPEIMKSNLESIEFDLSEEDIATISAFDRGLRFNQPTNYFPTEHLWIFG

SEQ ID NO: 2 - DNA, 978 bp, Thermochaetoides thermophila
  source 1..978: mol_type = genomic DNA
atggctccccagatccccaacattaagctcagcagcggctatgacatgccccaggtgggctttggactgtggaaggtcgaccgctcgatctgcgccgacgtcgtctacaacgcaattaagattggctaccgcctgtttgacggcgcttgcgactatggcaacgaagtcgaggccggccagggcattgcccgcgccatcaaggagggcatcgtgaagcgtgaggagctcttcatcgtgtccaagctctggaacaccttccacgacggcgacaaggtcgagcccatcgtccgcaagcagctcgccgactggggcattgactacttcgacctctacctcgtccacttccctgtcgccctcgagtacgtcgacccctcggtccgctacccgcccggctggttctacgatggcgagaaggagatccgccccagcaaggccaccatccaggagacctggaccgccatggagtcgctcgttgagaagggtctggcccgcagcattggtgtctccaacttccaggcccagctcctctacgacctgctgcgctacgccaagatccgcccggccacccttcagatcgagcatcaccccttcctcgtccagcaggagctgctcaacctggccaaggccgagggcattgccgtgactgcctacagctcattcggccctcagagcttcctcgagttcaacatgaagcacgccgtgcagctcaccccgctcttcgaggacgagaccatcaagaagatcgccgccaagtacaaccgtcctgcttcgcaggttctcctgcgctgggccactcagcgcggtctggccattatccccaagagcacgcgccccgagatcatgaagtccaacctcgagagcatcgagttcgacctcagcgaggaagatattgccaccatctcggccttcgaccgcggcctgcgcttcaaccagcccacaaactacttccccaccgagcacctctggatctttggctaa

SEQ ID NO: 3 - protein, 320 aa, Rasamsonia emersonii
MATPTIKLNSGYDMPLVGFGLWKVNKETCADQVYEAIKAGYRLFDGACDYGNEVEAGQGVARAIKEGIVKREDLFIVSKLWNTFHEADKVEPIARKQLADWGLDYFDLYLIHFPIALKYVDPAEIYPPGWTGTKKEVEFSNATIQETWQAMETLVDKKLTRSIGISNFSAQLIMDLLRYARIRPATLQIEHHPYLTQQALVEYVQKEGIAVTAYSSFGPLSFLELGHQVAKDTPLLFEHSTVKSIAEKHGKTPAQVLLRWATQRNIAVIPKSNNPGRLAQNLDVTAWDLEPADIEALSALNKNLRFNNPPSYGLYIPIFA

SEQ ID NO: 4 - DNA, 963 bp, Rasamsonia emersonii
  source 1..963: mol_type = genomic DNA
atggccacgcctactatcaagctgaacagcggctatgacatgcccctggtgggctttggtctgtggaaggtcaacaaggaaacctgcgcggaccaggtctacgaggctatcaaggcgggctaccgcttgtttgacggtgcgtgcgactatggcaacgaagttgaggccggccagggtgtcgctcgcgccatcaaggaaggcattgtgaagcgtgaggacctcttcattgtgtccaagctgtggaacacgttccacgaggccgacaaggtcgagccgatcgcgcggaagcagctggccgactggggcctcgactactttgacctgtacctcatccacttcccgatcgcgctgaagtacgtcgacccggccgagatctacccgccgggctggacgggcaccaagaaggaggtcgagttcagcaacgcgacgatccaggagacgtggcaggccatggagaccctggtcgacaagaagctgacgcgcagcatcggcatcagcaacttcagcgcccagctgatcatggacctgctgcggtacgcgcgcatccgccccgcgaccttgcagatcgagcaccacccgtacctgacgcagcaggcgctggtcgagtacgtgcagaaggagggcatcgccgtgacggcgtactcgtccttcggcccactgagcttcctggaactgggccaccaggtcgccaaggacacgccgctgctcttcgagcactcgaccgtcaagtcgatcgccgagaagcacggcaagacgcccgcccaggtgctactgcgctgggccacccagcgcaacatcgccgtcatccccaagagcaacaacccgggccgcctggcgcagaacctggacgtgacggcgtgggatctggagcccgccgacattgaggccttgagcgcgctgaacaagaaccttcgattcaacaacccacctagctacggactgtacatcccgatcttcgcttaa

SEQ ID NO: 5 - protein, 322 aa, Chaetomium globosum
MAPVIKLNSGYDMPQVGFGLWKVDNAVASDVVYNAIKAGYRLFDGACDYGNEVECGQGVARAISEGIVKREDLFIVSKLWNTFHDAERVEPIVKKQLADWGIEYFDLYLIHFPVALEWVDPAVRYPPGWHYDGKEEIRPSKATIQETWTALESLVSKGLSKSIGISNFQAQLIYDLLRYAKIRPATLQVEHHPYLVQQELINLAKREGIAVTAYSSFGPASFKEFNMKHADALAPLIEDETIKKIAAKHNRPASQVLLRWATQRGLAIIPKSTRPQIMAENFQSIDFDLSEEDIATISAFDRGIRFNQPSNYFPTELLWIFG

SEQ ID NO: 6 - DNA, 969 bp, Chaetomium globosum
  source 1..969: mol_type = genomic DNA
atggcgccggtgattaaactgaacagcggctatgatatgccgcaggtgggctttggcctgtggaaagtggataacgcggtggcgagcgatgtggtgtataacgcgattaaagcgggctatcgcctgtttgatggcgcgtgcgattatggcaacgaagtggaatgcggccagggcgtggcgcgcgcgattagcgaaggcattgtgaaacgcgaagatctgtttattgtgagcaaactgtggaacacctttcatgatgcggaacgcgtggaaccgattgtgaaaaaacagctggcggattggggcattgaatattttgatctgtatctgattcattttccggtggcgctggaatgggtggatccggcggtgcgctatccgccgggctggcattatgatggcaaagaagaaattcgcccgagcaaagcgaccattcaggaaacctggaccgcgctggaaagcctggtgagcaaaggcctgagcaaaagcattggcattagcaactttcaggcgcagctgatttatgatctgctgcgctatgcgaaaattcgcccggcgaccctgcaggtggaacatcatccgtatctggtgcagcaggaactgattaacctggcgaaacgcgaaggcattgcggtgaccgcgtatagcagctttggcccggcgagctttaaagaatttaacatgaaacatgcggatgcgctggcgccgctgattgaagatgaaaccattaaaaaaattgcggcgaaacataaccgcccggcgagccaggtgctgctgcgctgggcgacccagcgcggcctggcgattattccgaaaagcacccgcccgcagattatggcggaaaactttcagagcattgattttgatctgagcgaagaagatattgcgaccattagcgcgtttgatcgcggcattcgctttaaccagccgagcaactattttccgaccgaactgctgtggatttttggctaa

SEQ ID NO: 7 - protein, 324 aa, Candida tropicalis
MSTTVNTPTIKLNSGYEMPLVGFGCWKVTNATAADQIYNAIKTGYRLFDGAEDYGNEKEVGEGINRAIKDGLVKREELFITSKLWNNFHDPKNVETALNKTLSDLNLDYVDLFLIHFPIAFKFVPIEEKYPPGFYCGDGDNFHYEDVPLLDTWKALEKLVEAGKIKSIGISNFTGALIYDLIRGATIKPAVLQIEHHPYLQQPKLIEYVQKAGIAITGYSSFGPQSFLELESKRALNTPTLFEHETIKSIADKHGKSPAQVLLRWATQRNIAVIPKSNNPERLAQNLSVVDFDLTKDDLDNIAKLDIGLRFNDPWDWDNIPIFV

SEQ ID NO: 8 - DNA, 974 bp, Candida tropicalis
  source 1..974: mol_type = genomic DNA
atgagcacgaccgttaatactccgacgatcaaactgaactccggttacgagatgccgctggttggctttggctgttggaaagttaccaatgcgacggcggcggaccagatttataacgctattaaaaccggttaccgtctgttcgatggcgcagaggactacggtaacgagaaagaagtgggtgaaggtattaatcgcgcaattaaagacggtctggtcaaacgtgaagagctgtttattacctcgaaactgtggaataacttccatgatcctaagaacgtggagactgcgctgaataagaccctgagcgatctgaacctggactatgtggatctgtttctgattcacttcccgattgctttcaaatttgtcccgatcgaagaaaagtacccaccgggcttctactgcggtgacggcgacaacttccattatgaggatgttccgctgctggacacgtggaaggcgctggagaaattggtggaagccggtaagatcaagtccattggcattagcaacttcaccggtgccttgatttacgatttgatccgtggtgcgaccattaaaccggcggttctgcagatcgagcatcacccgtatctgcaacagccgaaactgatcgaatacgttcagaaagcaggtatcgccatcactggctatagcagcttcggtccacagagcttcctggagctggagagcaagcgtgccctgaataccccgacgttgtttgaacacgaaaccatcaagtctatcgctgacaaacacggtaagagccctgcacaagtcctgctgcgctgggcaacgcaacgtaatattgcggttattccgaagagcaataacccggagcgtctggcgcagaatctgtctgtcgtcgactttgatttgaccaaggatgacctggataatatcgcgaagctggacatcggcctgcgcttcaacgatccgtgggattgggacaacatcccgatctttgtgta

SEQ ID NO: 9 - protein, 329 aa, Kluyveromyces lactis
MTYLAETVTLNNGEKMPLVGLGCWKMPNDVCADQIYEAIKIGYRLFDGAQDYANEKEVGQGVNRAIKEGLVKREDLVVVSKLWNSFHHPDNVPRALERTLSDLQLDYVDIFYIHFPLAFKPVPFDEKYPPGFYTGKEDEAKGHIEEEQVPLLDTWRALEKLVDQGKIKSLGISNFSGALIQDLLRGARIKPVALQIEHHPYLTQERLIKYVKNAGIQVVAYSSFGPVSFLELENKKALNTPTLFEHDTIKSIASKHKVTPQQVLLRWATQNGIAIIPKSSKKERLLDNLRINDALTLTDDELKQISGLNQNIRFNDPWEWLDNEFPTFI

SEQ ID NO: 10 - DNA, 990 bp, Kluyveromyces lactis
  source 1..990: mol_type = genomic DNA
atgacgtacttagcagaaacagttactttaaacaatggcgaaaagatgccgctagtcggcttaggttgctggaagatgcccaacgacgtttgtgccgaccaaatttacgaagccattaagatcggatatcgtttattcgatggtgcccaagattacgccaacgagaaagaagttggacagggtgtcaacagagccatcaaagaagggcttgttaagagagaggatttagttgttgtctccaagctatggaacagtttccaccatccggacaacgtacctcgtgctttggaaagaactctttccgatttgcaattggactatgttgacatattctacatccatttcccattggccttcaagcctgtgccattcgatgagaagtatcctccaggtttctacaccggtaaggaagacgaagctaaaggtcacattgaagaagaacaagtaccactattggacacttggagggctttagaaaaactagtcgaccaaggtaagatcaagtccttgggtatttccaacttttcaggtgcgttgatccaagatttgctacgtggtgctcgtatcaagccagttgccctacaaatcgagcatcatccatatttgacacaggaaagattgattaaatacgtcaagaatgccggcattcaagtggttgcctactcctcgttcggtccagtgtcgttcctggaattggaaaacaagaaagctcttaacacccctactttgtttgagcatgacacgattaagtctatcgcttccaagcacaaagtcactccacaacaagttctgttgagatgggccacacaaaatggcattgccatcattccaaaatcatcaaagaaggaaagattgctggataacttgaggatcaacgatgcattgactttgaccgatgatgaattgaagcaaatttccggcttgaatcaaaatatcagattcaatgacccttgggaatggctagacaacgaattcccaactttcatctaa

SEQ ID NO: 11 - protein, 323 aa, Thermothelomyces thermophilus
MPSPVIKLNSGYDMPQVGFGLWKVDNSVAADVVYNAIKAGYRLFDGACDYGNEVECGKGIARAISEGIVKREDLFIVSKLWNTFHDAERVEPIVKKQLADWGIDYFDLYLIHFPVALEYVDPSVRYPPGWFYDGKSEIRTSKATIQETWTAMESLVAKGLTKSIGISNFQAQLIYDLLRYAKIRPATLQIEHHPYLVQQELLNLAKQEGIAVTAYSSFGPASFLEFNMQHAVKLTPLIEDETIKKIAAKYNREPAQVLLRWATQRGLAVIPKTTRPALMASNFQCTDFDLSEEDIATISSFDRGIRFNQPSNYFPTEYLWIFG

SEQ ID NO: 12 - DNA, 972 bp, Thermothelomyces thermophilus
  source 1..972: mol_type = genomic DNA
atgccgtcacctgtcatcaagctcaacagcggctatgacatgccccaggtgggcttcggcctctggaaggtcgacaattccgttgccgcggacgtcgtctacaacgccatcaaggccggctaccgcctcttcgatggcgcttgcgactacggcaacgaggtcgagtgcggcaagggtatcgcgcgcgccatctcggagggcattgtgaagcgtgaggacctcttcatcgtgtccaagctctggaacaccttccacgacgccgagcgcgtcgagcccatcgtcaagaagcagctcgccgactggggcattgactacttcgacctctacctcatccacttccctgtcgccctcgagtacgtcgacccctcggtccgctacccgcccggttggttctacgatggcaagagcgagatccgcaccagcaaggccaccatccaggagacctggactgccatggagtcccttgtcgccaagggcctcaccaagagcatcggtatttccaacttccaggcccagctgatctacgacctcctgcggtacgccaagatccgcccggccaccctccagatcgagcaccacccctacctcgtccagcaggagctgctcaacctcgccaagcaggagggcatcgccgtcaccgcctacagctccttcggccccgccagcttcctcgagttcaacatgcagcacgccgtcaagctcaccccccttatcgaggacgagaccatcaagaagatcgccgccaagtacaaccgcgagcccgcccaagtcctgctccgctgggccactcagcgtggcctggccgtcatccccaagaccacccgccccgccctcatggcctccaacttccagtgcaccgactttgatctctccgaggaggacatcgccaccatctcgtccttcgaccgcggcattcgcttcaaccagccctccaactacttccccaccgagtatctctggatctttggctaa

SEQ ID NO: 13 - protein, 332 aa, Gluconobacter frateurii
MSTDTILIPGIDTPVSRVALGTWAIGGWMWGGPDDGNGVRTIHAALDDGINLIDTAPVYGFGHSEEVVGRALAEKPHKAFVATKLGLNWTDDKPEDRKVFRDSRPARIRQEVEDSLRRLRVETIDLEQIHWPDAKTPIDESARELQKLHQEGKIRALGVSNFSPEQMDIFREVAPLATIQPPLNLFERTCEKDILPYAKKNDAVVLAYGSLCRGLLSGKMSKDTTFPKDDLRSGDPKFQKPKFESYLAAVEDFKKLAAKRNKSVLAFAVRWVLDQGPVIALWGARKPEQVSGVRDVFGWSLTDEEKKAVDEILAHHVPEAIDPTFMGPPNRD

SEQ ID NO: 14 - DNA, 999 bp, Gluconobacter frateurii
  source 1..999: mol_type = genomic DNA
atgtccaccgacaccattctcattccaggcattgatacgcccgtttctcgcgttgcccttggcacctgggctatcggtggctggatgtggggcggccctgacgatggaaacggcgtccgcaccattcatgccgcccttgatgatggcatcaatctgattgataccgctccggtttacggctttggacattccgaagaagttgtgggtcgcgcactggctgagaagccgcacaaggcctttgtcgccacaaagctgggcctgaactggacggatgacaagccggaagaccggaaggtctttcgtgactcccgccccgcccgtatccgacaggaagtggaagactccctgcgccgcctgcgcgttgagacgatcgaccttgagcagattcactggccggatgccaagaccccgatcgacgaaagcgcgcgcgagcttcagaagctgcatcaggaaggcaagatccgcgctctgggcgtcagcaacttctcgcccgaacagatggatattttccgcgaagtcgcgcccctcgccacgatccagccgccgctgaacctgttcgagcgtacctgtgaaaaggacatcctgccgtacgcgaagaagaacgatgcggttgttctggcctatggttcgctatgtcgcggtctgctgtccggcaaaatgagcaaggacacgacgttcccgaaggatgatctgcgttcgggtgatccgaaattccagaagccgaagttcgagagctatctggccgctgtcgaggacttcaagaagctggctgccaagcggaacaagtccgttctcgcctttgctgtccgctgggtactggatcagggaccggtcattgctctctggggcgctcgcaagccggagcaggtctcaggcgtacgagacgttttcggctggtctctgacggatgaagaaaagaaggccgtagacgaaattctggcgcatcatgtgccggaggccatcgacccgacctttatggggccgccgaaccgcgactaa

SEQ ID NO: 15 - protein, 332 aa, Gluconobacter cerinus
MSSDTILIPGIDTPVSRVALGTWAIGGWMWGGPDDENGVRTIHAALDDGINFIDTAPVYGFGHSEEVVGRALAEKPNKAFVATKLGLNWTDDKPEDRKVFRDSRPARIRKEVEDSLRRLRVETIDLEQIHWPDDKTPIDESARELQKLHQEGKIRALGVSNFSPEQMDIFREVAPLATIQPPLNLFERTCEKDILPYAKKNNAVVLAYGALCRGLLSGKMNKDTSFPKDDLRSGDPKFQKPKFESYLAAVEDFKELAAKRDKSVLAFAVRWVLDQGPVIALWGARKPEQVSGVKDVFGWSLTDEEKKAVDEILARHVPDAIDPTFMGPPNRD

SEQ ID NO: 16 - DNA, 999 bp, Gluconobacter cerinus
  source 1..999: mol_type = genomic DNA
atgtcctcagacaccattctcattcccggcatcgacactccggtttcccgcgtggctctcggcacctgggccattggcggctggatgtggggcgggccggacgatgaaaacggcgttcgcaccatccatgcagctctcgatgacggcatcaatttcatcgacacggcacccgtctatggcttcgggcactcagaagaagttgttggccgggcactggccgaaaagcccaacaaggctttcgttgcgacaaagctgggcctgaactggacggatgacaaacccgaagaccgcaaggttttccgtgattcccgccctgcccgcatccgcaaggaagtggaagactccctgcgccgcctgcgggtcgaaacgattgatctcgaacagatccattggcccgatgacaagactcccatcgatgaaagcgcacgcgagctgcagaaacttcatcaggaaggcaagatccgggcgctcggcgttagcaatttctcgccggagcagatggatatctttcgcgaagtcgccccactcgcaacaattcagcccccgctgaacctgttcgaacgcacctgcgaaaaagatattctcccatacgccaagaagaataacgccgtggtgctcgcttatggcgcgctctgccgcggactgctctccggcaagatgaacaaggatacgagcttcccgaaagatgacctgcgttcaggtgatccgaagttccagaagccaaagttcgagagctatctcgccgcagtcgaagacttcaaggagctggccgccaagcgcgacaagtccgttctcgccttcgctgtacgctgggttctggatcaggggccagtcatcgcactctggggcgcacgcaagcctgaacaggtctccggcgtgaaggatgttttcggctggtctctgaccgacgaagaaaagaaggctgtggacgaaattctggcacgtcacgtcccggacgcgatcgacccgaccttcatggggccaccgaaccgcgactaa

SEQ ID NO: 17 - protein, 327 aa, Saccharomyces cerevisiae
MSSLVTLNNGLKMPLVGLGCWKIDKKVCANQIYEAIKLGYRLFDGACDYGNEKEVGEGIRKAISEGLVSRKDIFVVSKLWNNFHHPDHVKLALKKTLSDMGLDYLDLYYIHFPIAFKYVPFEEKYPPGFYTGADDEKKGHITEAHVPIIDTYRALEECVDEGLIKSIGVSNFQGSLIQDLLRGCRIKPVALQIEHHPYLTQEHLVEFCKLHDIQVVAYSSFGPQSFIEMDLQLAKTTPTLFENDVIKKVSQNHPGSTTSQVLLRWATQRGIAVIPKSSKKERLLGNLEIEKKFTLTEQELKDISALNANIRFNDPWTWLDGKFPTFA

SEQ ID NO: 18 - DNA, 984 bp, Saccharomyces cerevisiae
  source 1..984: mol_type = genomic DNA
atgtcttcactggttactcttaataacggtctgaaaatgcccctagtcggcttagggtgctggaaaattgacaaaaaagtctgtgcgaatcaaatttatgaagctatcaaattaggctaccgtttattcgatggtgcttgcgactacggcaacgaaaaggaagttggtgaaggtatcaggaaagccatctccgaaggtcttgtttctagaaaggatatatttgttgtttcaaagttatggaacaattttcaccatcctgatcatgtaaaattagctttaaagaagaccttaagcgatatgggacttgattatttagacctgtattatattcacttcccaatcgccttcaaatatgttccatttgaagagaaataccctccaggattctatacgggcgcagatgacgagaagaaaggtcacatcaccgaagcacatgtaccaatcatagatacgtaccgggctctggaagaatgtgttgatgaaggcttgattaagtctattggtgtttccaactttcagggaagcttgattcaagatttattacgtggttgtagaatcaagcccgtggctttgcaaattgaacaccatccttatttgactcaagaacacctagttgagttttgtaaattacacgatatccaagtagttgcttactcctccttcggtcctcaatcattcattgagatggacttacagttggcaaaaaccacgccaactctgttcgagaatgatgtaatcaagaaggtctcacaaaaccatccaggcagtaccacttcccaagtattgcttagatgggcaactcagagaggcattgccgtcattccaaaatcttccaagaaggaaaggttacttggcaacctagaaatcgaaaaaaagttcactttaacggagcaagaattgaaggatatttctgcactaaatgccaacatcagatttaatgatccatggacctggttggatggtaaattccccacttttgcctaa